European Patent Application EP 4 737 587 A1, published May 6, 2026. Title: 利用封闭子进行纳米孔测序的方法. Applicant: 深圳华大生命科学研究院. The sequence listing filed with the application follows.

SEQUENCE LISTING (15 sequences)

SEQ ID NO: 1 - DNA, 39 bp, synthetic construct
  source 1..39: mol_type = other DNA
  modified_base 1..10: mod_base = OTHER; note = Int C3 Spacer
  modified_base 21..24: mod_base = OTHER; note = Int Spacer 18
nnnnnnnnnnttttttttttnnnnggttgtttctgttgg

SEQ ID NO: 2 - DNA, 49 bp, synthetic construct
  source 1..49: mol_type = other DNA
  modified_base 1..20: mod_base = OTHER; note = Int C3 Spacer
  modified_base 31..34: mod_base = OTHER; note = Int Spacer 18
nnnnnnnnnnnnnnnnnnnnttttttttttnnnnggttgtttctgttgg

SEQ ID NO: 3 - DNA, 59 bp, synthetic construct
  source 1..59: mol_type = other DNA
  modified_base 1..30: mod_base = OTHER; note = Int C3 Spacer
  modified_base 41..44: mod_base = OTHER; note = Int Spacer 18
nnnnnnnnnnnnnnnnnnnnnnnnnnnnnnttttttttttnnnnggttgtttctgttgg

SEQ ID NO: 4 - DNA, 33 bp, synthetic construct
  source 1..33: mol_type = other DNA
ccaacagaaacaacctttgaggcgagcggtcaa

SEQ ID NO: 5 - DNA, 19 bp, synthetic construct
  source 1..19: mol_type = other DNA
  modified_base 1..4: mod_base = OTHER; note = Int Spacer 18
nnnnttgaccgctcgcctc

SEQ ID NO: 6 - protein, 442 aa, synthetic construct
GSHGTFDDLTEGQKNAFNIVMKAIKEKKHHVTINGPAGTGKTTLTKFIIEALISTGETGIILAAPTHAAKKILSKLSGKEASTIHSILKINPVTYECNVLFEQKEVPDLAKARVLICDEVSMYDRKLFKILLSTIPPWATIIGIGDNKQIRPVDPGENTAYISPFFTHKDFYQCELTEVKRSNAPIIDVATDVRNGLWIYDKVVDGHGVRGFTGDTALRDFMVNYFSIVKSLDDLFENRVMAFTNKSVDKLNSIIRKKIFETDKDFIVGEIIVMQEPLFKTYKIDGKPVSEIIFNNGQLVRIIEAEYTSTFVKARGVPGEYLIRHWDLTVETYGDDEYYREKIKIISSDEELYKFNLFLGKTCETYKNWNKGGKAPWSDFWDAKSQFSKVKALPASTFHKAQGMSVDRAFIYTPCIHYADVELAQQLLYVGVTRGRYDVFYV

SEQ ID NO: 7 - DNA, 72 bp, synthetic construct
  source 1..72: mol_type = other DNA
  modified_base 1..30: mod_base = OTHER; note = Int C3 Spacer
  modified_base 41..44: mod_base = OTHER; note = Int Spacer 18
nnnnnnnnnnnnnnnnnnnnnnnnnnnnnnttttttttttnnnnggttgtttctgttggtgctgatattgct

SEQ ID NO: 8 - skipped

SEQ ID NO: 9 - RNA, 15 nt, synthetic construct
  source 1..15: mol_type = other RNA
ccaacagaaacaacc

SEQ ID NO: 10 - DNA, 35 bp, synthetic construct
  source 1..35: mol_type = other DNA
  modified_base 26..35: mod_base = OTHER; note = Int C3 Spacer
gaggcgagcggtcaattttttttttnnnnnnnnnn

SEQ ID NO: 11 - DNA, 45 bp, synthetic construct
  source 1..45: mol_type = other DNA
  modified_base 26..45: mod_base = OTHER; note = Int C3 Spacer
gaggcgagcggtcaattttttttttnnnnnnnnnnnnnnnnnnnn

SEQ ID NO: 12 - DNA, 55 bp, synthetic construct
  source 1..55: mol_type = other DNA
  modified_base 26..55: mod_base = OTHER; note = Int C3 Spacer
gaggcgagcggtcaattttttttttnnnnnnnnnnnnnnnnnnnnnnnnnnnnnn

SEQ ID NO: 13 - DNA, 33 bp, synthetic construct
  source 1..33: mol_type = other DNA
aatgcctaagtactgaaattgaccgctcgcctc

SEQ ID NO: 14 - DNA, 19 bp, synthetic construct
  source 1..19: mol_type = other DNA
  modified_base 16..19: mod_base = OTHER; note = Int Spacer 18
cagtacttaggcattnnnn

SEQ ID NO: 15 - DNA, 45 bp, synthetic construct
  source 1..45: mol_type = other DNA
gcaatatcagcaccaacagaaacaacctttgaggcgagcggtcaa